European Patent Specification EP 3 969 600 B1, published August 7, 2024. Title: ENZYMATIC PRODUCTION OF GLUCARIC ACID FROM GLUCURONIC ACID. Applicant: THE GOVERNING COUNCIL OF THE UNIVERSITY OF TORONTO. The sequence listing filed with the application follows.

SEQUENCE LISTING (5 sequences)

SEQ ID NO: 1 - protein, 474 aa, Sarocladium strictum
  MISC_FEATURE (1)..(206): FAD-binding domain
  MISC_FEATURE (207)..(474): substrate-binding domain
NSINACLAAADVEFHEEDSEGWEMDGTAFNLRVDYDPVAIAIPRSTEDIAAAVQCGLDAGVQISAKGGGHSYGSYGFGGEDGHLMLELDRMYRVSVDDDNVATIQGGARLGYTALELLDQGNRALTHGTCPAVGIGGHVLGGGYGFATHTHGLTLDWLVGATVVLADASIVHVSKTENADLFWALRGGGGGFAIVSEFEFNTFEAPEIITTYQVTTTWNRKQHVAGLKALQDWAENTMPRELSMRLEINANALNWEGNYFGNAKDLKKVLQPIMKKAGGKSTISKLVETDWYGQINTYLYGADLNITYNYDVHEYFYANSLTAPRLSDEAISAFVDYKFDNSSVRPGRGWWIQWDFHGGKNSALASHSNDETAYAHRDQLWLWQFYDNIYDYENNTSPYPESGFEFMQGFVATIEDTLPEDRKGKYFNYADTTLDKEEAQKLYWRGNLEKLQAIKAKYDPEDVFGNVVSVEPIA

SEQ ID NO: 2 - protein, 206 aa, Sarocladium strictum
  MISC_FEATURE (1)..(206): FAD-binding domain of SEQ ID NO: 1
NSINACLAAADVEFHEEDSEGWEMDGTAFNLRVDYDPVAIAIPRSTEDIAAAVQCGLDAGVQISAKGGGHSYGSYGFGGEDGHLMLELDRMYRVSVDDDNVATIQGGARLGYTALELLDQGNRALTHGTCPAVGIGGHVLGGGYGFATHTHGLTLDWLVGATVVLADASIVHVSKTENADLFWALRGGGGGFAIVSEFEFNTFEAP

SEQ ID NO: 3 - protein, 268 aa, Sarocladium strictum
  MISC_FEATURE (1)..(268): substrate-binding domain of SEQ ID NO: 1
EIITTYQVTTTWNRKQHVAGLKALQDWAENTMPRELSMRLEINANALNWEGNYFGNAKDLKKVLQPIMKKAGGKSTISKLVETDWYGQINTYLYGADLNITYNYDVHEYFYANSLTAPRLSDEAISAFVDYKFDNSSVRPGRGWWIQWDFHGGKNSALASHSNDETAYAHRDQLWLWQFYDNIYDYENNTSPYPESGFEFMQGFVATIEDTLPEDRKGKYFNYADTTLDKEEAQKLYWRGNLEKLQAIKAKYDPEDVFGNVVSVEPIA

SEQ ID NO: 4 - protein, 966 aa, Amphibacillus xylanus
MDFTLNQEMLMTDTKSGALFYQEEEALSGVRKIANKVMHDVELVFGYQPEATKDRDMLSRHAVLYGTVGHSPLLDELNKKELIDLTEIAGKREVFLFQVVDQPIQGVEKALVIAGSDKRGTIYGLFHLSEKLGVSPLVDWSGVLPARKESFSLKGDYKYVSKEPSVKYRGFFINDEWPAFGNWSAKNFGGFNAEMYDHVFELLLRLKGNYLWPAMWSARFNDDGPGLANVELADEYGVIMGASHHEPCLRYGEEYKYLRGPDSIYGDAWNFITNREGITKFWEDGLKRTGHFENIITIGMRGEADTKIMGEDATLEDNINLLRDVIQTQNKLIKEHVNPNLKEVPRMLALYKEVEPFFYGDENTPGLINSEELEDVILMLCDDNHGNLRTLPTEDMRKHSGGYGMYYHFDYHGGPVSYEWINSSYLPKIWEQMTMAYDFGVRDLWIVNVGDIATQELPLSFFLDLAYDFDKWGTNAINKTDDYTKQWIEQQFAGVFNLEQKDKVFELLNGYTKIAHNRRPEAMNVDVYHPVNYHETDQLLDRIDHLLGLAEELYQEVDQQHFTAYFALVYYPTVGNLNLQKMWLLNGKNKYAAQLNLIEANKLAEQVKACLKRDQEIVDEYHTIADGKFYGMGLSEHIGFVHWNEDENKNPVLSYVLPVNKPRLLVSIDGTELRSEGSPWHVNTLPLVDFLEPDVNQASFTISSVSEKKAEYHISTDQDWLSCSAANGVLDGKNKLSETIHVFVDRDGLADQAEGRITVKTPVGKVTIVVPVVNNDFTNYPDMTFVDTKGYISIEAEHFATQKATENLDGTLNRFEVLDGYGKTLSAIKAFPTDTHYQVGKDAPFVEYHFVTQEAGVYELEFYLQPSNPVTREGTMYAGIQVNENDVDVINVLPDGYHVDGPHWGIDVINNIRTTKTKITCEQGLNKLRIYAVSPGFALEKIVIYPDGKKLANSYLGPNETYYVGR

SEQ ID NO: 5 - protein, 943 aa, Saccharophagus degradans 2-40
VLALGDAGYISFKANGGVRLADEEHLASLLVDTNDYKGLQRAAADLQTDMQRVTGKLPTLHSQLKDAGRHAVIIGSVGRSGLIQLLVEQNKLNVADIEGQWEAYKLVVVDKPFPNIEKALVIAGSDMRGAIFGVYDLSQQIGVSPWYWWADVPVQPQSKLYVRGDTHIVEQPKVQYRGIFLNDEAPALTNWVHANYGNYNSQFYTQVFELLLRLKANFLWPAMWNNSFSVDDPLNPVLANEYGIVMSTSHHEPMMRAHKEWHGMGRWDFTTNADALKQFWREGVERNSPYENIITMAMRGDGDEAMSEDANVELLEQIVEAQRNIIAEVFEPKGKQVTEVPQVWCLYKEVQDYYEKGMRVPDDITLLWADDNWGNIRRLPTAEERKRSGGAGVYYHFDYVGGPRSYRWINTTPLAKIWEQMHLAYKYEANKIWIVNVGDLKPMEAPIEYFLEMAWNPEQWPKERITQFAELWAEREFGPTYAKEIAQLVQDYTQHNGRRKPELQEAKTYSLLNYDEAARIEQQLTDMESRAETLFNKIPANQRDAYYQLVMHPVLASATVTKMYIAQARNRLYAKQGRPIANSYGQQVKELFEKDAALTKRYHSINNGKWNHFMSQPHIGYTHWNNPEDNIMPVVSVVSKGNNADMGVAVEGMEPAWPTQDVAFALPTFTPYGKQTKILTVFNKGVKPLKFSVSSGAAWLKVSASSGEITHQEMQIQVSIDWAKLPLGIHESNVTIKGPSWVAANIKVTANKPAKVIPLKKLTGFVEADGYISFDAAATTHSKAVDGFEWQEIPAHGRTHSSMSVYPIRDASFAAPANASANTAPQMHYSITLLTAGEVTVEGLFAPTWPIHPERGLRYAIAFDDQPPQIVDVLAGNSHKVWQESVRTGVRRASSKHTLTAGTHTMKVWAIDPAVTVQKWIIDTGELKPSYLGPTPSPRGGKH